European Patent Specification EP 4 039 282 B1, published June 4, 2025. Title: Nucleic acid inhibiting expression of MEX3B gene, MEX3B gene expression inhibitor, method for inhibiting MEX3B gene expression, and prophylactic or therapeutic agent for disease caused by MEX3B gene expression. Applicant: THE UNIVERSITY OF TOKYO. The sequence listing filed with the application follows.

SEQUENCE LISTING (34 sequences)

SEQ ID NO: 1 - DNA, 16 bp, Artificial Sequence
  hmrGD-89-2
gcggatactacagctt

SEQ ID NO: 2 - DNA, 16 bp, Artificial Sequence
  hmrGD-89
gagcggatactacagc

SEQ ID NO: 3 - DNA, 14 bp, Artificial Sequence
  common
gcggatactacagc

SEQ ID NO: 4 - DNA, 3532 bp, Human
tcaagaggcggggaggagaggaggaaaaagcgctgagtgagggcgggcgggcgggcgggagggagggagtggaggagccggggaggggctccttaaagaaacgcttctgtcgctcgcctgctcgcttttcgctcggcattgcggccagccagccgggcactcggggggcacgcgcggccaccgctagagctctgcccccaccccacccgccagcaggtctggggtggggacccaggtgggggctcctgcagccactgcccggtgcggaccgcacggagcgacccactcctcccagcaccgaggaagaagcaacggagccctcagcaggcgaccggcctccccgcccctgaccacccgcttcccggctgcctttgtggccgcagcttctcgccgccgagccgagggccggcgggggcgcggcgcgcacggccgagcgatgcccagctcgctgttcgcagacctggagcgcaacggcagcggcggcggcggcggcggcagcagcggagggggagagaccctggatgaccaaagagccctgcagctcgcgctcgaccagctctccctgctggggctggacagtgacgagggcgcctctctgtacgacagcgagccgcgcaagaagagcgtgaacatgaccgagtgcgtgccagtacccagttctgagcatgtcgccgagatcgtggggcggcaaggttgtaaaatcaaagcgctgcgggcgaagaccaatacttacatcaagaccccagttcgcggggaggagcctgtctttgttgtgacgggcaggaaggaggatgtggccatggctcggagggagatcatctctgctgccgagcacttctccatgatccgcgcctcccggaataagaacacggcactcaacggcgcggtgcctgggccgcccaacctgcccgggcagaccaccatccaagtgcgggtaccctaccgcgtggtggggctcgtggtggggcccaaaggcgccacaatcaagcgcatccagcagcagacgcacacgtacatcgtgacgcccagccgggataaggagccggtgttcgaggtgaccggcatgccagagaacgtggatcgcgctcgagaggagattgaggcgcacattgctctgcgtaccggcggcatcattgagctcacagacgagaacgacttccacgccaacggcaccgatgtgggcttcgatctgcatcatgggtccggcgggtccggcccaggcagcctctggagcaagcccacccccagcatcacgcccacccccggccgcaagcctttctctagctaccgcaacgacagctccagctcgcttggcagtgcttccacagactcttatttcggcggcgggaccagcagcagcgcagcggctacccagcgcctggcggactacagcccccctagccccgccctgagctttgcgcacaacggaaacaataacaataacggcaatgggtacacctacacagcggggggagaagcctcagtgccatcccccgacggctgccccgagctgcagcccacttttgacccggctcccgctcccccacctggggcaccacttatctgggcccagttcgagcggtccccgggaggcggacctgcagctccggtatcttcttcctgctcttcttctgcatcttcgtctgcttcttcctcctccgtggtcttccccgggggtggcgccagtgcgccctccaacgccaacctggggctattggtgcaccgccggctgcaccctggcaccagctgcccgcgcctgtctccacccttgcacatggccccgggggcgggagagcaccacctggctcgccgggtgcgcagcgacccgggtggaggaggcctggcctacgccgcttatgccaacgggctgggggcacagctgcctggcttgcagccgtcggacacgtcgggctcctcctcttcgtccagctcctcctccagctcttcatcctcttcctccgggcttcggcgtaaaggcagccgcgactgctccgtgtgcttcgagagcgaagtgattgccgcgctggtgccctgtggccacaacctcttctgcatggagtgcgccaatcgcatctgtgagaagagcgagcccgagtgcccggtctgccacaccgcggtcactcaggccatccgcatcttttcttaaaggcagcgggcgctgctagtgcgcaccgtgctgggggaagggggaacccctccccatcctctttccccagcgctcgcctgcctccctgggtgccccccctctcccttctccttcccggccccaccaacactctgagatccgagaggagcttggaaagctgtagtatccgctcatttttaaaatttaatttttaagtaaaggaatttgccaggatatctgcatcaagagtactgtagcctgggaaacctgaacacctgaaatgcatgctctataaataataggaacggcgacattctagtaatgatagtttttacactgtacttaataggaagcttccaaaagaagaaaaccccacaagttttccattttcttaaagtaggaaaaaatgaacagtaataattatgatgaagatgatagtagtgctatgggatgtgtggactgtttagtgtgttcccctttgtgggtgggttcctatgatacttattatagaacacagtggatcctttttgaatgttcgtggaagggccaggagttcctgtgaaaccaggatactgcagctttattaaagttaaagaaactgtaacatatctcttatatattaaaaacgtttaaaagttttaaagagaaattgcattaatacagattgaagtattttattcttttttgacttgaaaaattatatttcatattgcaaagatgtttacaagtattttaatttaagttcagtgaacttttttgtagctgggttaaatctttttattttagtatggccttatggcaaagaacactgtattattttaataatcacacaattgtgacggaattacaaccataaaatgtgtaatgttttgaacagtattctgttgggatggagattttataggttcagacaaatcttctagatctgcttcacccagcatattttctattcagtgatataaagcatattttattctatattattacaaaaacggaaatgtataaacatgtcaaaaagaactgttgatgctttctaacatttgtataaatagaattcagtgcaagttacaaaaattctgttgcaccactctagttttagtatttctattttaatacatttgtttaccacttgtttatgtatatgtaggtgatgttacttgagcttaaatgtactttactgagcaaagtttaaaaaacaaagtatattttattttatgataaagggcctttaacctcatggtcaaatactaatattatatttgctgagacaagatttgaaattgtatcaagagttttatttttctgacatttaaagttctacataataaaggtaaaacttaagtaatggtgctacttcattttttaagtatttctatataaataaaatattgaagaaaatcttaaaaa

SEQ ID NO: 5 - DNA, 3416 bp, Mouse
tgttcgctttgcgctcggcattgtggccagccagccgggcactcggggggcacgcgcggccgccgctcgagctctgcccccaccccaaccgccagcagatctggggtggggacccaggcgggggctcttgcagccactgcccggtgcggattgcacgcagagacccactcctccgagcgccgaaaaacgagccacggagccctccgcagccgaccggcctccccgcccctgactgccggcttcccggctgcctttgtggctgcaccttctagctgccgagcagagagccggctggggcgcggcgcgcacggcggagcgatgcccagctcgctgtttgcagacctggagcgcaacggcagcggcggcggcgggggaggcggcggcgggggaggcggcggtggcagcggcgggggagagactctggatgaccaaagagccctgcagcttgcgctcgatcagctctccctgttgggactggacagtgatgagggcgcctctttgtacgacagcgaaccgcgcaagaagagcgtgaacatgaccgagtgcgtgccggtacccagttccgaacacgtcgcggagatcgtagggaggcaaggttgtaaaatcaaagctttgagggcgaagaccaacacttacatcaagaccccagttcgcggggaggagcctgtctttgttgtgacgggcaggaaggaggatgtggctatggctcggagggagatcatctctgccgcagagcacttctccatgatccgagcctctcgtaacaagaacacggctctcaacggagctgtgcccggaccgcccaacctgccgggacagaccactatccaagtgagggtgccataccgcgtggtagggctcgtggtgggtccaaagggcgccacgatcaagcgcattcaacagcagacacatacatatattgtgacacccagccgagacaaggagccagttttcgaggtgactggcatgccagagaacgtggatcgcgctagagaggagatcgaagctcacatcgcgctgcgcaccggtggcatcatcgagctgacagacgagaacgacttccatgccaatggcacagacgtgggctttgatctgcatcacgggtccggcgggtccgggccgggcagcctctggagcaagcccaccccaagcatcactcctacacctggccgcaagcccttctccagctatcgcaacgacagctccagctcgcttggcagcgcatccacagactcttacttcggtggtgggaccagcggcagcgcagctgctacttcacgcctggcggactatagccctcccagccctgcactcagctttgctcacaatgggaacaacaacaataacggcaatggttacacctacacagcgggggaagcctcagtaccttccccagatgggggtcctgagctgcagcctactttcgacccagctcccgccccaccacctgggacaccccttctctgggcccagttcgagcgctctccaggaggtggatctgcagcaccagtatcctcttcctgctcttcttcggcatcctcatctgcctcgtcgtcctctgtggtctttcccgggggtggcgccagcagcacaccctccaatgccaatctggggctgctggtgcaccgtcgactgcacccgggcaccagctgcccgcgcctgtctccgcccttgcacatggccacgggggcgggagagcaccaccttgctcgccgcgtgcgcagcgacccgggcggtggaggcctggcctacgctgcctatgctaatgggctagggacgcagctccctggcctgccctcgtcggacacttcgggctcctcctcgtcctctagctcctcctccagctcttcctcctcttcctctgggctgaggcgcaaaggcagccgcgactgctctgtgtgcttcgagagtgaagtgatcgccgcgctggtgccctgtggccacaacctcttctgcatggagtgtgccaaccgcatttgtgagaagagcgagcccgagtgtcccgtctgccacacggcggtcactcaggccatccgcattttttcctgaaggcagtgcgcgcgcgcgcactgcagggaaggagggtcctctctcgaccctcattccctagggtctacctgcccagacgcctctggtgcccacctctttccaccccaccctcatcactctcagagatcccagaggagcttggaaagctgtagtatccgctcatttttaaaatgtcatttttaaacaaaggaacttgccaggatctctgcatcaggagtactgtagcctccgaaccacctgaattgcatgctctataaataataggaacggcgacattctagtaacgatagtttttacactgtacttaataggaagcttccaaaagaaaaccccacaagttttccattttcttgaagtagaaaaatgaacagtaattatgaagatgattaataattgtgctatgggatgtgtggactgttttgtgtgtttccctttgtgggtgggttcctacagcgctcgttctagaacacaagtggatcctttttgaatgttcatggaagggccaggagttctgtacagccaggaccctgcagctttattaaagttaaaactgtaacatatctcttatatattaaaaaaaaaaacctttaaaagttttaaagagaaattgcattaatacagattgaagtattttattctttttttgacttgaaaaattatatttcatattgcaaagatgtttacaagtattttaatttaagttcagtgaacttttttgtagctgggttaaatctttttatttttagtatggccttatggcaaagaacactgtattattttaataatcacacgattgtgacggattacaaaccataaaatgtataacgttttgagcagtattctgttgggatggagattttataggttcagacaaatcttctagatctgcttcacccagcatattttctattcagtgatataaagcatattttattctatattattacaaaaaatggaaatgtataaacatgtcaaaaggaacagttgatgctttctaacatttgtataaatagaattcagtgcaaattacagaaattctgttgcaccgctatagttttagtgtttctattttaatacatttgtttaccactcgtttatgtatatgtaggtgacgttacttgagcttaaatgtactttactgagcaaagtttaaaaaaaaacaaagtatattttattttatgataaagggcctttaacctcatggtcaaatactaatattatatttgctgagacaagatttgaaattgtatcaagagttttatttttctgacatttaaagttctacataataaaggtaaacttaagtaatggtgctacttcattttttaagtatttctatataaataaaacattgaagaaaaatcact

SEQ ID NO: 6 - DNA, 836 bp, Human
gtaggtcgaggagggatggggaggtgggtgggggtggtgtagggtctcaggccactgcctcgaggggaaggcgtgttcagtatcgggatccgcggcgtggggtgccttggggagagaggaagagccgcgcgatgggccggcgccccagacaaagaaagtgcaggcaggctgtctcccggagccgcgccgctgccctggcgggatgcactttcttctgctaaaatcactgccttctcccctaacgccccccaaccagcccacctccagaaagacaatttaaatgtaagatgcttgggggagggggcctttgatcagtcctttgggaggaggaaggaggaggagtgagcataggatgggaggaggattctggatttctgcaaagcggaatggagcccagaggaggaacaatgggtcccgggactcacaccccaccccctacccccagtcgaccagcgctgaggcatcgcgacttcagctgccttccccgagccccttccccgtgtcttcagagctgacggcgcgcccagctggatcccagcggcatctccccagatgacttttctgggattctcgggtttggttcgggacgactgcagtcactgggggagggccaggcagccaatgggctgttcctcgagcgcctcgcgggtgggatccgctgcccagcccgtggcgcggcccgaggtcagtgagggagacgccccctttccgcccatctcttgtcctgccgtctcgctgtcctggacgcgggctgtccccggtccccgcggttaccccaggataatgggcgtgtctgtctctctctcccactccctcctccgcaccctggttcgtag

SEQ ID NO: 7 - DNA, 4368 bp, Human
tcaagaggcggggaggagaggaggaaaaagcgctgagtgagggcgggcgggcgggcgggagggagggagtggaggagccggggaggggctccttaaagaaacgcttctgtcgctcgcctgctcgcttttcgctcggcattgcggccagccagccgggcactcggggggcacgcgcggccaccgctagagctctgcccccaccccacccgccagcaggtctggggtggggacccaggtgggggctcctgcagccactgcccggtgcggaccgcacggagcgacccactcctcccagcaccgaggaagaagcaacggagccctcagcaggcgaccggcctccccgcccctgaccacccgcttcccggctgcctttgtggccgcagcttctcgccgccgagccgagggccggcgggggcgcggcgcgcacggccgagcgatgcccagctcgctgttcgcagacctggagcgcaacggcagcggcggcggcggcggcggcagcagcggagggggagagaccctggatgaccaaagagccctgcagctcgcgctcgaccagctctccctgctggggctggacagtgacgagggcgcctctctgtacgacagcgagccgcgcaagaagagcgtgaacatgaccgagtgcgtgccagtacccagttctgagcatgtcgccgagatcgtggggcggcaaggtaggtcgaggagggatggggaggtgggtgggggtggtgtagggtctcaggccactgcctcgaggggaaggcgtgttcagtatcgggatccgcggcgtggggtgccttggggagagaggaagagccgcgcgatgggccggcgccccagacaaagaaagtgcaggcaggctgtctcccggagccgcgccgctgccctggcgggatgcactttcttctgctaaaatcactgccttctcccctaacgccccccaaccagcccacctccagaaagacaatttaaatgtaagatgcttgggggagggggcctttgatcagtcctttgggaggaggaaggaggaggagtgagcataggatgggaggaggattctggatttctgcaaagcggaatggagcccagaggaggaacaatgggtcccgggactcacaccccaccccctacccccagtcgaccagcgctgaggcatcgcgacttcagctgccttccccgagccccttccccgtgtcttcagagctgacggcgcgcccagctggatcccagcggcatctccccagatgacttttctgggattctcgggtttggttcgggacgactgcagtcactgggggagggccaggcagccaatgggctgttcctcgagcgcctcgcgggtgggatccgctgcccagcccgtggcgcggcccgaggtcagtgagggagacgccccctttccgcccatctcttgtcctgccgtctcgctgtcctggacgcgggctgtccccggtccccgcggttaccccaggataatgggcgtgtctgtctctctctcccactccctcctccgcaccctggttcgtaggttgtaaaatcaaagcgctgcgggcgaagaccaatacttacatcaagaccccagttcgcggggaggagcctgtctttgttgtgacgggcaggaaggaggatgtggccatggctcggagggagatcatctctgctgccgagcacttctccatgatccgcgcctcccggaataagaacacggcactcaacggcgcggtgcctgggccgcccaacctgcccgggcagaccaccatccaagtgcgggtaccctaccgcgtggtggggctcgtggtggggcccaaaggcgccacaatcaagcgcatccagcagcagacgcacacgtacatcgtgacgcccagccgggataaggagccggtgttcgaggtgaccggcatgccagagaacgtggatcgcgctcgagaggagattgaggcgcacattgctctgcgtaccggcggcatcattgagctcacagacgagaacgacttccacgccaacggcaccgatgtgggcttcgatctgcatcatgggtccggcgggtccggcccaggcagcctctggagcaagcccacccccagcatcacgcccacccccggccgcaagcctttctctagctaccgcaacgacagctccagctcgcttggcagtgcttccacagactcttatttcggcggcgggaccagcagcagcgcagcggctacccagcgcctggcggactacagcccccctagccccgccctgagctttgcgcacaacggaaacaataacaataacggcaatgggtacacctacacagcggggggagaagcctcagtgccatcccccgacggctgccccgagctgcagcccacttttgacccggctcccgctcccccacctggggcaccacttatctgggcccagttcgagcggtccccgggaggcggacctgcagctccggtatcttcttcctgctcttcttctgcatcttcgtctgcttcttcctcctccgtggtcttccccgggggtggcgccagtgcgccctccaacgccaacctggggctattggtgcaccgccggctgcaccctggcaccagctgcccgcgcctgtctccacccttgcacatggccccgggggcgggagagcaccacctggctcgccgggtgcgcagcgacccgggtggaggaggcctggcctacgccgcttatgccaacgggctgggggcacagctgcctggcttgcagccgtcggacacgtcgggctcctcctcttcgtccagctcctcctccagctcttcatcctcttcctccgggcttcggcgtaaaggcagccgcgactgctccgtgtgcttcgagagcgaagtgattgccgcgctggtgccctgtggccacaacctcttctgcatggagtgcgccaatcgcatctgtgagaagagcgagcccgagtgcccggtctgccacaccgcggtcactcaggccatccgcatcttttcttaaaggcagcgggcgctgctagtgcgcaccgtgctgggggaagggggaacccctccccaccctctttccccagcgctcgcctgcctccctgggtgccccccctctcccttctccttcccggccccaccaacactctgagatccgagaggagcttggaaagctgtagtatccgctcatttttaaaatttaatttttaagtaaaggaatttgccaggatatctgcatcaagagtactgtagcctgggaaacctgaacacctgaaatgcatgctctataaataataggaacggcgacattctagtaatgatagtttttacactgtacttaataggaagcttccaaaagaagaaaaccccacaagttttccattttcttaaagtaggaaaaaatgaacagtaataattatgatgaagatgatagtagtgctatgggatgtgtggactgtttagtgtgttcccctttgtgggtgggttcctatgatacttattatagaacacagtggatcctttttgaatgttcgtggaagggccaggagttcctgtgaaaccaggatactgcagctttattaaagttaaagaaactgtaacatatctcttatatattaaaaacgtttaaaagttttaaagagaaattgcattaatacagattgaagtattttattcttttttgacttgaaaaattatatttcatattgcaaagatgtttacaagtattttaatttaagttcagtgaacttttttgtagctgggttaaatctttttattttagtatggccttatggcaaagaacactgtattattttaataatcacacaattgtgacggaattacaaccataaaatgtgtaatgttttgaacagtattctgttgggatggagattttataggttcagacaaatcttctagatctgcttcacccagcatattttctattcagtgatataaagcatattttattctatattattacaaaaacggaaatgtataaacatgtcaaaaagaactgttgatgctttctaacatttgtataaatagaattcagtgcaagttacaaaaattctgttgcaccactctagttttagtatttctattttaatacatttgtttaccacttgtttatgtatatgtaggtgatgttacttgagcttaaatgtactttactgagcaaagtttaaaaaacaaagtatattttattttatgataaagggcctttaacctcatggtcaaatactaatattatatttgctgagacaagatttgaaattgtatcaagagttttatttttctgacatttaaagttctacataataaaggtaaaacttaagtaatggtgctacttcattttttaagtatttctatataaataaaatattgaagaaaatcttaaaaa

SEQ ID NO: 8 - protein, 569 aa, Human
MPSSLFADLERNGSGGGGGGSSGGGETLDDQRALQLALDQLSLLGLDSDEGASLYDSEPRKKSVNMTECVPVPSSEHVAEIVGRQGCKIKALRAKTNTYIKTPVRGEEPVFVVTGRKEDVAMARREIISAAEHFSMIRASRNKNTALNGAVPGPPNLPGQTTIQVRVPYRVVGLVVGPKGATIKRIQQQTHTYIVTPSRDKEPVFEVTGMPENVDRAREEIEAHIALRTGGIIELTDENDFHANGTDVGFDLHHGSGGSGPGSLWSKPTPSITPTPGRKPFSSYRNDSSSSLGSASTDSYFGGGTSSSAAATQRLADYSPPSPALSFAHNGNNNNNGNGYTYTAGGEASVPSPDGCPELQPTFDPAPAPPPGAPLIWAQFERSPGGGPAAPVSSSCSSSASSSASSSSVVFPGGGASAPSNANLGLLVHRRLHPGTSCPRLSPPLHMAPGAGEHHLARRVRSDPGGGGLAYAAYANGLGAQLPGLQPSDTSGSSSSSSSSSSSSSSSSGLRRKGSRDCSVCFESEVIAALVPCGHNLFCMECANRICEKSEPECPVCHTAVTQAIRIFS

SEQ ID NO: 9 - protein, 576 aa, Mouse
MPSSLFADLERNGSGGGGGGGGGGGGGGSGGGETLDDQRALQLALDQLSLLGLDSDEGASLYDSEPRKKSVNMTECVPVPSSEHVAEIVGRQGCKIKALRAKTNTYIKTPVRGEEPVFVVTGRKEDVAMARREIISAAEHFSMIRASRNKNTALNGAVPGPPNLPGQTTIQVRVPYRVVGLVVGPKGATIKRIQQQTHTYIVTPSRDKEPVFEVTGMPENVDRAREEIEAHIALRTGGIIELTDENDFHANGTDVGFDLHHGSGGSGPGSLWSKPTPSITPTPGRKPFSSYRNDSSSSLGSASTDSYFGGGTSGSAAATSRLADYSPPSPALSFAHNGNNNNNGNGYTYTAGEASVPSPDGGPELQPTFDPAPAPPPGTPLLWAQFERSPGGGSAAPVSSSCSSSASSSASSSSVVFPGGGASSTPSNANLGLLVHRRLHPGTSCPRLSPPLHMATGAGEHHLARRVRSDPGGGGLAYAAYANGLGTQLPGLPSSDTSGSSSSSSSSSSSSSSSSGLRRKGSRDCSVCFESEVIAALVPCGHNLFCMECANRICEKSEPECPVCHTAVTQAIRIFS

SEQ ID NO: 10 - DNA, 15 bp, Artificial Sequence
  control
aacacgtctatacgc

SEQ ID NO: 11 - DNA, 16 bp, Artificial Sequence
  hmrGD-87
tacagctttccaagct

SEQ ID NO: 12 - DNA, 16 bp, Artificial Sequence
  hmrGD-88
gatactacagctttcc

SEQ ID NO: 13 - DNA, 16 bp, Artificial Sequence
  hmrGD-90
aaaatgagcggatact

SEQ ID NO: 14 - DNA, 16 bp, Artificial Sequence
  hmrGD-91
atttatagagcatgca

SEQ ID NO: 15 - DNA, 16 bp, Artificial Sequence
  hmrGD-92
ctattatttatagagc

SEQ ID NO: 16 - DNA, 16 bp, Artificial Sequence
  hmrGD-93
cgttcctattatttat

SEQ ID NO: 17 - DNA, 16 bp, Artificial Sequence
  hmrGD-176
gtacatttaagctcaa

SEQ ID NO: 18 - DNA, 16 bp, Artificial Sequence
  hmrGD-178
gctcagtaaagtacat

SEQ ID NO: 19 - DNA, 16 bp, Artificial Sequence
  hmrGD-179
actttgctcagtaaag

SEQ ID NO: 20 - DNA, 16 bp, Artificial Sequence
  hmrGD-180
tttaaactttgctcag

SEQ ID NO: 21 - DNA, 16 bp, Artificial Sequence
  hmrGD-182
cataaaataaaatata

SEQ ID NO: 22 - DNA, 16 bp, Artificial Sequence
  hmrGD-199
aaaaataaaactcttg

SEQ ID NO: 23 - DNA, 16 bp, Artificial Sequence
  hmrGD-201
taaatgtcagaaaaat

SEQ ID NO: 24 - DNA, 16 bp, Artificial Sequence
  hmrGD-202
aactttaaatgtcaga

SEQ ID NO: 25 - DNA, 16 bp, Artificial Sequence
  hmrGD-203
tgtagaactttaaatg

SEQ ID NO: 26 - DNA, 16 bp, Artificial Sequence
  hmrGD-205
acctttattatgtaga

SEQ ID NO: 27 - DNA, 20 bp, Artificial Sequence
  primer
acccagttctgagcatgtcg

SEQ ID NO: 28 - DNA, 21 bp, Artificial Sequence
  primer
cgaactggggtcttgatgtaa

SEQ ID NO: 29 - DNA, 20 bp, Artificial Sequence
  GAPDH primer 2 F
gcaccgtcaaggctgagaac

SEQ ID NO: 30 - DNA, 19 bp, Artificial Sequence
  Human GAPDH primer 2 Reverse
tggtgaagacgccagtgga

SEQ ID NO: 31 - DNA, 30 bp, Artificial Sequence
  MEX3B primer Fw1
cgtcgtcctctgtggtctttcccgggggtg

SEQ ID NO: 32 - DNA, 30 bp, Artificial Sequence
  MEX3B primer Rv1
tcaggaaaaaatgcggatggcctgagtgac

SEQ ID NO: 33 - DNA, 22 bp, Artificial Sequence
  Mouse B-actin primerFw
ggatgcagaaggagattactgc

SEQ ID NO: 34 - DNA, 20 bp, Artificial Sequence
  Mouse B-actin primerRv
ccaccgatccacacagagca